European Patent Specification EP 3 726 218 B1, published August 9, 2023. Title: CELL LINES FOR SCREENING ODORANT AND AROMA RECEPTORS. Applicant: Firmenich SA. The sequence listing filed with the application follows.

SEQUENCE LISTING (20 sequences)

SEQ ID NO: 1 - DNA, 21 bp, artificial
  Guide RNA target sequence
ctgcaatctcagttcagggcc

SEQ ID NO: 2 - DNA, 3628 bp, artificial
  Donor DNA for homology directed repair
ggggttttatggaagagtcttacttctcttttctttcatctatattttgtattttttctagaataaacccatatgattttttaaaaggaaaaataatttattaaaaatagcagcagaggcatgtatagtaaaggctgttttgcctgtgggtggtgctcctcttctgcgcttctataatcagcttggaaataatcttgtctgctcctgcctggctgatgcaatgctcctacctttgtgcacaggtggctgttcttgcacaaggccattgcagcatggatcctattgcacagttattcagtacacagtcagctacaagcactgacatagagcttggcacatgtctgcaaaccctacccacatgctcggatatgtttgaaatgaatgaattaatgaaccggtctggggtcaacagcttgaatttgtatacaggctccgccatttataggctaggtgagtcctaggctcctgatctgtactgcagcaatagtaatcataacttaagagacctccaattgtgttttgaaaatggcaaagtgctggtcacaagatggctggggaagccgagagagagtttattattattgctccatctactaacaaatttacatctccccatccctcatttctccttggctgcctaaggcatcatggttaccgtagcagccagatgctgatgatgcctccaggggacggcaaggtgaaactgagccagttcccagtcctcacctccccatactctttccaggccagggtgagatggtctgaagctcagtctctggtcaggtcccccactctgtcttggatcatttagacccgcggccgcggcgcgcctcggaattcgattgaagttcctattccgaagttcctattctctagaaagtataggaacttcggtgtggaaagtccccaggctccccagcaggcagaagtatgcaaagcatgcatctcaattagtcagcaaccatagtcccgcccctaactccgcccatcccgcccctaactccgcccagttccgcccattctccgccccatggctgactaattttttttatttatgcagaggccgaggccgcctcggcctctgagctattccagaagtagtgaggaggcttttttggaggcctaggcttttgcaaaaagcttgcatgcctgcaggtcggccgccacgaccggtgccgccaccatcccctgacccacgcccctgacccctcacaaggagacgaccttccatgaccgagtacaagcccacggtgcgcctcgccacccgcgacgacgtcccccgggccgtacgcaccctcgccgccgcgttcgccgactaccccgccacgcgccacaccgtcgacccggaccgccacatcgagcgggtcaccgagctgcaagaactcttcctcacgcgcgtcgggctcgacatcggcaaggtgtgggtcgcggacgacggcgccgcggtggcggtctggaccacgccggagagcgtcgaagcgggggcggtgttcgccgagatcggcccgcgcatggccgagttgagcggttcccggctggccgcgcagcaacagatggaaggcctcctggcgccgcaccggcccaaggagcccgcgtggttcctggccaccgtcggcgtctcgcccgaccaccagggcaagggtctgggcagcgccgtcgtgctccccggagtggaggcggccgagcgcgccggggtgcccgccttcctggagacctccgcgccccgcaacctccccttctacgagcggctcggcttcaccgtcaccgccgacgtcgaggtgcccgaaggaccgcgcacctggtgcatgacccgcaagcccggtgcctgacgcccgccccacgacccgcagcgcccgaccgaaaggagcgcacgaccccatggctccgaccgaagccacccggggcggccccgccgaccccgcacccgcccccgaggcccaccgactctagaggatcataatcagccataccacatttgtagaggttttacttgctttaaaaaacctcccacacctccccctgaacctgaaacataaaatgaatgcaattgttgttgttaacttgtttattgcagcttataatggttacaaataaagcaatagcatcacaaatttcacaaataaagcatttttttcactgcgaagttcctattccgaagttcctattctctagaaagtataggaacttcaatcactagtgaattcacgcgttgacattgattattgactagttattaatagtaatcaattacggggtcattagttcatagcccatatatggagttccgcgttacataacttacggtaaatggcccgcctggctgaccgcccaacgacccccgcccattgacgtcaataatgacgtatgttcccatagtaacgccaatagggactttccattgacgtcaatgggtggagtatttacggtaaactgcccacttggcagtacatcaagtgtatcatatgccaagtacgccccctattgacgtcaatgacggtaaatggcccgcctggcattatgcccagtacatgaccttatgggactttcctacttggcagtacatctacgtattagtcatcgctattaccatggtgatgcggttttggcagtacatcaatgggcgtggatagcggtttgactcacggggatttccaagtctccaccccattgacgtcaatgggagtttgttttggcaccaaaatcaacgggactttccaaaatgtcgtaacaactccgccccattgacgcaaatgggcggtaggcgtgtacggtgggaggtctatataagcagagctcgtttagtgaaccgtgtttaaacctcttcagagactccctcctccccaagctctgtcttctggcaacctgcctggttgccgtggaaacaggttccactgcggacaaaggagggagctgggtcctgcttcctcctggtcttgtcgatgaggatttttagaccgtggagactgcgctgccctgccctgcacctaccctcactctccgtgttctcactaaggtggaaattgccttccctcactactgacgagaccatgtgtaaaagcgtgaccacagatgagtggaagaaagtcttctatgagaagatggaggaggcaaagccggctgacagctgggacctcatcatagaccccaacctcaagcacaatgtgctgagccctggttggaagcagtacctggaattgcatgcttcaggcaggtgagtagcccaggaaagtggatccctgcaggccgcctctaggtccctagctctggggcaccttccaaggagaggaagattacgtagaacccaagtgtttagcttcaatctcactattaggctggcgtagactggaagtcagagaaagagtccctaactgggaactacgacacttgagttggatttcagctcttctactgatcacctgtgttactcttcctctctgagtcacaatttttccgtctggaaaataaagacatagaatatacgtatgagtcctacacactgacattttacatattttctattttaacagtctcttaaaaagtagtttaaaaccagagaagaagggtttgaggcccactgggggtcgagacgtccgtgctctggtcctgggaccggtttaaatctatttaa

SEQ ID NO: 3 - DNA, 928 bp, mouse
atgaaaaccctcagcagccccagcaactccagcaccatcactggcttcatcctcttgggcttcgcctaccccagggaggggcaaattctcctctttgtgatcttcttcattgtttacatactcattcttatgggcaacgcttccatcatctgtgctgtgtactgtgatcagagactccacacccccatgtaccttctgctggccaacttctccttcatggagattggatatgtcacctccacagtccccaacatgttggccaacttcctttcagacaccaaggtcatctctttctctggatgcttcctgcagttctatttcttcttctcctttggttctacagaatgctttttcctggcagtcatggcatttgatcgataccttgccatctgtaggccactacattatccttctctcatgactgggcgcctccgaaacacccttgtgaccagttgctgggtgcttggtttcctctggttccctgtacccatcatcatcatctcccagatgtccttctgtgggtccagaattatagaccacttcctgtgtgacccaggccctcttttggcccttgcctgttccagagtcccattgatagaggttttctggtccattataatgtctatgctcctggttattcctttcctcttcatcatgggaacttacatattggtcctaagagctgtgtttagacttccttcaagagaaggacaaaaaaaggctttctccacttgcgggtctcatctcacagtagtttcactcttttattgctcagtgatgataatgtatctgagcccaacatctgagcatgaggccggaatgcagaagcttgtaactctattttattctgtgggtacaccactgcttaatcctatgatatacagtctgaggaacaaagatatgaaaaatgccctacagaagattttga

SEQ ID NO: 4 - protein, 311 aa, mouse
MKTLSSPSNSSTITGFILLGFAYPREGQILLFVIFFIVYILILMGNASIICAVYCDQRLHTPMYLLLANFSFMEIGYVTSTVPNMLANFLSDTKVISFSGCFLQFYFFFSFGSTECFFLAVMAFDRYLAICRPLHYPSLMTGRLRNTLVTSCWVLGFLWFPVPIIIISQMSFCGSRIIDHFLCDPGPLLALACSRVPLIEVFWSIIMSMLLVIPFLFIMGTYILVLRAVFRLPSREGQKKAFSTCGSHLTVVSLFYCSVMIMYLSPTSEHEAGMQKLVTLFYSVGTPLLNPMIYSLRNKDMKNALQKILRT

SEQ ID NO: 5 - DNA, 936 bp, mouse
atgaaaaccctcagcagccccagcaactccagcaccatcactggcttcatcctcttgggcttcccctgccccagggaggggcaaatcctcctctttgtgaccttcttcattgtttacatactcattcttatgggcaatgcttccatcatctgtgctgtgtactgtgatcagagcctccacacccccatgtacttcctgctggccaacttctccttcctggagatctggtatgtcacctccacagtccccaacatgttggccaacttcctttcagacaccaaggtcatctctttctctggatgcttcctgcagttctatttcttcttctcctttggttctacagaatgctttttcctggcagtcatggcatttgatcgataccttgccatctgtaggccactacattatccttctctcatgactgggcacctctgcaacatccttgtgatcagttgctgggtgcttggtttcctctggttccctgtacccatcatcatcatctcccagatgtccttctgtgggtccagaattatagaccacttcctgtgtgacccaggccctcttttggcccttgcctgttccagagccccattgatggaggttttctggacaattataatgtctatgctcctggttattcctttcctcttcatcatgggaacttacatattggtcctaagagctgtgtttagacttccttcaagagatggacaaaaaaaggccttctccacttgcgggtctcatctcacagtagtttcactcttttattgctcagtgatgaaaatgtatttgagcccaacatctgagcatgaagctggaatgcagaagcttgtaactctattttattctgtgggtactccactacttaatcctgtgatatacagtctgaggaacaaagatatgaaaaatgccctgcagaagattttaagaacataa

SEQ ID NO: 6 - protein, 311 aa, mouse
MKTLSSPSNSSTITGFILLGFPCPREGQILLFVTFFIVYILILMGNASIICAVYCDQSLHTPMYFLLANFSFLEIWYVTSTVPNMLANFLSDTKVISFSGCFLQFYFFFSFGSTECFFLAVMAFDRYLAICRPLHYPSLMTGHLCNILVISCWVLGFLWFPVPIIIISQMSFCGSRIIDHFLCDPGPLLALACSRAPLMEVFWTIIMSMLLVIPFLFIMGTYILVLRAVFRLPSRDGQKKAFSTCGSHLTVVSLFYCSVMKMYLSPTSEHEAGMQKLVTLFYSVGTPLLNPVIYSLRNKDMKNALQKILRT

SEQ ID NO: 7 - DNA, 942 bp, mouse
atgggaatcctttccacaggaaatcaaactgtcactgagtttgtacttcttggtttccatgaagtccctgggctgcacctcctgtttttttctgtgttcaccatcctctatgcctccatcatcacagggaacatgctcattgcagtggtggtggtgagctcccagaggcttcacacacccatgtatttctttctggtgaatctgtccttcatagagattgtctatacctccacagtggtgcccaaaatgctggaaggcttcttacaggaggccaccatatctgtggctggctgcttgctccagttctttgtttttggctctctggccacagatgagtgttttctgctggctgtgatggcatatgatcgatatctcgcaatttgtcaccctctacgatacccacacctcatggggcctcaatggtgcctggggttggtgctcacagtctggctgtctggcttcatggtagatggactagttgttgctctgatggcccagttgagattctgtggccccaacttagttgatcacttttactgtgatttttcacctttgatggtcctggcttgctcagatacccaagtggcccaggtgactacatttgttctctctgtggtcttcctgactgtcccctttgggctggttctgatctcctatgctcagattgtagtgactgtgctgagagttccttctgggaccagaagaaccaaggccttctccacatgctcctctcacctggctgtggtgtccacgttctatggaacactcatggtattgtacattgtgccctctgctgttcattctcagctcctctccaaggtcattgccctgctctacacagtggtcactcccatcttcaaccctgtcatctacaccttgaggaaccaggaggtgcagcaggcactaagaaggcttctctactgcaaaccaactgaaatgtga

SEQ ID NO: 8 - protein, 313 aa, mouse
MGILSTGNQTVTEFVLLGFHEVPGLHLLFFSVFTILYASIITGNMLIAVVVVSSQRLHTPMYFFLVNLSFIEIVYTSTVVPKMLEGFLQEATISVAGCLLQFFVFGSLATDECFLLAVMAYDRYLAICHPLRYPHLMGPQWCLGLVLTVWLSGFMVDGLVVALMAQLRFCGPNLVDHFYCDFSPLMVLACSDTQVAQVTTFVLSVVFLTVPFGLVLISYAQIVVTVLRVPSGTRRTKAFSTCSSHLAVVSTFYGTLMVLYIVPSAVHSQLLSKVIALLYTVVTPIFNPVIYTLRNQEVQQALRRLLYCKPTEM

SEQ ID NO: 9 - DNA, 948 bp, human
atggaaattgtctccacaggaaacgaaactattactgaatttgtcctccttggcttctatgacatccctgaactgcatttcttgttttttattgtattcactgctgtctatgtcttcatcatcatagggaatatgctgattattgtagcagtggttagctcccagaggctccacaaacccatgtatattttcttggcgaatctgtccttcctggatattctctacacctccgcagtgatgccaaaaatgctggagggcttcctgcaagaagcaactatctctgtggctggttgcttgctccagttctttatcttcggctctctagccacagctgaatgcttactgctggctgtcatggcatatgaccgctacctggcaatttgctacccactccactacccactcctgatggggcccagacggtacatggggctggtggtcacaacctggctctctggatttgtggtagatggactggttgtggccctggtggcccagctgaggttctgtggccccaaccacattgaccagttttactgtgactttatgcttttcgtgggcctggcttgctcggatcccagagtggctcaggtgacaactctcattctgtctgtgttctgcctcactattccttttggactgattctgacatcttatgccagaattgtggtggcagtgctgagagttcctgctggggcaagcaggagaagggctttctccacatgctcctcccacctagctgtagtgaccacattctatggaacgctcatgatcttttatgttgcaccctctgctgtccattcccagctcctctccaaggtcttctccctgctctacactgtggtcacccctctcttcaatcctgtgatctataccatgaggaacaaggaggtgcatcaggcacttcggaagattctctgtatcaaacaaactgaaacacttgattga

SEQ ID NO: 10 - protein, 315 aa, human
MEIVSTGNETITEFVLLGFYDIPELHFLFFIVFTAVYVFIIIGNMLIIVAVVSSQRLHKPMYIFLANLSFLDILYTSAVMPKMLEGFLQEATISVAGCLLQFFIFGSLATAECLLLAVMAYDRYLAICYPLHYPLLMGPRRYMGLVVTTWLSGFVVDGLVVALVAQLRFCGPNHIDQFYCDFMLFVGLACSDPRVAQVTTLILSVFCLTIPFGLILTSYARIVVAVLRVPAGASRRRAFSTCSSHLAVVTTFYGTLMIFYVAPSAVHSQLLSKVFSLLYTVVTPLFNPVIYTMRNKEVHQALRKILCIKQTETLD

SEQ ID NO: 11 - DNA, 936 bp, mouse
atgaaaaccttcagcagccccatcaactccagcaccaccactggcttcattctcttgggcttcccctgccccagggaggggcaaatcctcctctttgtgctcttctccattgtctacctgcttaccctcatgggcaacacttgcatcatctttgcagtatgctgggatcagagactccacacacccatgtacctactgctggccaacttctccttcctggagatctggtatgttacctccacagtccccaacatgttggccaatttcctctctgacaccaaggtcatctctttctctggatgcttcctgcagttctatttcttcttctccttgggttctacagaatgccttttcctggcagtcatggcatttgatcgataccttgccatctgtaggccactacattatcctgctctcatgactgggagcctctgcaacatccttgtgatcagttgctgggtgcttggtttcctctggttccctgttcccatcatcatcatctcccagatgtccttctgtgggtccagaattatagaccacttcctgtgtgacccaggccctctattggccctcacctgttccagagccccattaatggaggttttctggacaattataacatctcttatcctgttcgttcctttcctcttcatcatgggatcttatacattggtcctgagagctgtgttcagagttccttcaagagatggacaaaaaaaggctttctccacttgcggatctcatctcacagtagttttactcttttatggctcagtgatgataatgtatctaagcccgacctctgagcatgaagctggaatgcagaagcttgtgactctattttattctgtggttactccactcattaatcctgtgatatacagtctgaggaacaaggatatgaaacatgccctgcagaagattttaagaacataa

SEQ ID NO: 12 - protein, 311 aa, mouse
MKTFSSPINSSTTTGFILLGFPCPREGQILLFVLFSIVYLLTLMGNTCIIFAVCWDQRLHTPMYLLLANFSFLEIWYVTSTVPNMLANFLSDTKVISFSGCFLQFYFFFSLGSTECLFLAVMAFDRYLAICRPLHYPALMTGSLCNILVISCWVLGFLWFPVPIIIISQMSFCGSRIIDHFLCDPGPLLALTCSRAPLMEVFWTIITSLILFVPFLFIMGSYTLVLRAVFRVPSRDGQKKAFSTCGSHLTVVLLFYGSVMIMYLSPTSEHEAGMQKLVTLFYSVVTPLINPVIYSLRNKDMKHALQKILRT

SEQ ID NO: 13 - DNA, 930 bp, human
atgagggaaaataaccagtcctctacactggaattcatcctcctgggagttactggtcagcaggaacaggaagatttcttctacatcctcttcttgttcatttaccccatcacattgattggaaacctgctcatcgtcctagccatttgctctgatgttcgccttcacaaccccatgtattttctccttgccaacctctccttggttgacatcttcttctcatcggtaaccatccctaagatgctggccaaccatctcttgggcagcaaatccatctcttttgggggatgcctaacgcagatgtatttcatgatagccttgggtaacacagacagctatattttggctgcaatggcatatgatcgagctgtggccatcagccgcccacttcactacacaacaattatgagtccacggtcttgtatctggcttattgctgggtcttgggtgattggaaatgccaatgccctcccccacactctgctcacagctagtctgtccttctgtggcaaccaggaagtggccaacttctactgtgacattacccccttgctgaagttatcctgttctgacatccactttcatgtgaagatgatgtacctaggggttggcattttctctgtgccattactatgcatcattgtctcctatattcgagtcttctccacagtcttccaggttccttccaccaagggcgtgctcaaggccttctccacctgtggttcccacctcacggttgtctctttgtattatggtacagtcatgggcacgtatttccgccctttgaccaattatagcctaaaagacgcagtgatcactgtaatgtacacggcagtgaccccaatgttaaatcctttcatctacagtctgagaaatcgggacatgaaggctgccctgcggaaactcttcaacaagagaatctcctcgtga

SEQ ID NO: 14 - protein, 309 aa, human
MRENNQSSTLEFILLGVTGQQEQEDFFYILFLFIYPITLIGNLLIVLAICSDVRLHNPMYFLLANLSLVDIFFSSVTIPKMLANHLLGSKSISFGGCLTQMYFMIALGNTDSYILAAMAYDRAVAISRPLHYTTIMSPRSCIWLIAGSWVIGNANALPHTLLTASLSFCGNQEVANFYCDITPLLKLSCSDIHFHVKMMYLGVGIFSVPLLCIIVSYIRVFSTVFQVPSTKGVLKAFSTCGSHLTVVSLYYGTVMGTYFRPLTNYSLKDAVITVMYTAVTPMLNPFIYSLRNRDMKAALRKLFNKRISS

SEQ ID NO: 15 - DNA, 24 bp, artificial
  Flag tag
gattacaaggacgacgacgataag

SEQ ID NO: 16 - protein, 8 aa, artificial
  Flag tag
DYKDDDDK

SEQ ID NO: 17 - DNA, 60 bp, artificial
  Rho tag
atgaacgggaccgagggcccaaacttctacgtgcctttctccaacaagacgggcgtggtg

SEQ ID NO: 18 - protein, 20 aa, artificial
  Rho tag
MNGTEGPNFYVPFSNKTGVV

SEQ ID NO: 19 - DNA, 51 bp, artificial
  Lucy tag
atgagaccccagatcctgctgctcctggccctgctgaccctaggcctggct

SEQ ID NO: 20 - protein, 17 aa, artificial
  Lucy tag
MRPQILLLLALLTLGLA